European Patent Application EP 4 299 119 A1, published January 3, 2024. Title: Therapeutic applications based on the inhibition of G Protein-Coupled Receptor 182 (GPR182). Applicant: Max-Planck-Gesellschaft zur Förderung der Wissenschaften e.V. The sequence listing filed with the application follows.

SEQUENCE LISTING (3 sequences)

SEQ ID NO: 1 - RNA, 3411 nt, Homo sapiens
  #human GPR182 mRNA (NCBI Accession ID: NM_007264.4)
agcagtgacagctacttcccggatgagaagggcggccgtgaagccagcagggaagccagccccacagccaagggccccccagcctcctcacagctccccatagcctggacctgccggccctccctccaggaccgaggggctcccaagggaaactcaggcgtgtgctggtcccaatgtcagtgaaacccagctgggggcctggcccctcggagggggtcaccgcagtgcctaccagtgaccttggagagatccacaactggaccgagctgcttgacctcttcaaccacactttgtctgagtgccacgtggagctcagccagagcaccaagcgcgtggtcctctttgccctctacctggccatgtttgtggttgggctggtggagaacctcctggtgatatgcgtcaactggcgcggctcaggccgggcagggctgatgaacctctacatcctcaacatggccatcgcggacctgggcattgtcctgtctctgcccgtgtggatgctggaggtcacgctggactacacctggctctggggcagcttctcctgccgcttcactcactacttctactttgtcaacatgtatagcagcatcttcttcctggtgtgcctcagtgtcgaccgctatgtcaccctcaccagcgcctccccctcctggcagcgttaccagcaccgagtgcggcgggccatgtgtgcaggcatctgggtcctctcggccatcatcccgctgcctgaggtggtccacatccagctggtggagggccctgagcccatgtgcctcttcatggcaccttttgaaacgtacagcacctgggccctggcggtggccctgtccaccaccatcctgggcttcctgctgcccttccctctcatcacagtcttcaatgtgctgacagcctgccggctgcggcagccaggacaacccaagagccggcgccactgcctgctgctgtgcgcctacgtggccgtctttgtcatgtgctggctgccctatcatgtgaccctgctgctgctcacactgcatgggacccacatctccctccactgccacctggtccacctgctctacttcttctatgatgtcattgactgcttctccatgctgcactgtgtcatcaaccccatcctttacaactttctcagcccacacttccggggccggctcctgaatgctgtagtccattaccttcctaaggaccagaccaaggcgggcacatgcgcctcctcttcctcctgttccacccagcattccatcatcatcaccaagggtgatagccagcctgctgcagcagccccccaccctgagccaagcctgagctttcaggcacaccatttgcttccaaatacttcccccatctctcccactcagcctcttacacccagctgaggtagaggccagactcctccaacagtgaaggaaaaggcacaggtgagagtataggtgggagatttggggggatgtagaggggagggtcaaagcactcgtggtcaattttgaatctatcttaaaatactgaggtgtggagagagagacaggatcaggagcgatagagagcaggccctcagtgttgtactatttgtctcggtccttgtgtctaaggagcaatgcagaaaaaaaggtgaaataaatggaagagatagccatggactctggatcttttaaaaatctgcacttccagctgggattgggaagggagctgaggctaaagaggtgctcggcagaggaaactagacacattcatttcataaatcactctggctggaaacagtgaactctgcaggaacctcacaaaactccttttgcgtttgtgagcttgttgatcttccagctcactatgcaggttatggggacaagaggccagaggccaaggaaccaggcggccccagcaggacgttccctagctgtgcatcctatgcacagccatgataagtgaaggcggatggggatggcaggggtgggggcgaagccaaggtctgagacctgcaccctgcagctgggtcagcaggatggtatctccacccgcggccatccaggaaacacagctccatttccttgctgacaccctcccctccccgttgtccatcctgctccctccccacaagcaagaggagttgtcccagagtcagctcctcatagctgacctcttaccagcttcggatctaggaaacttccagacttctagggagacacagagctaccagaaagcccaacccacccccatctctttctctccagatcataggaaagtatcaagggatgtcattccgggagcagcccttgggacagccagcagcaggtgctggcagatgctctgtccttcaccctctgtccccggcaccagatggggaaggccacagtggaaacttctcaattccgtcacagggcagagctctgacactgttataagtcagttctccctggccatgtcttttcctaattttcctgtcccacaacttaggttccttaacacttgttctacagatgaaacaaaaaagtcctctgttaacaagtagaccttctggaaaaggatcacttatgtttgggagactaggaccctgtccatgaagaactctgaagtaaaggcctaagaacaggatctagtttccgccttccaattccacgtcctttgcctcttaatcctgcccgtggtaaggggactggatggaatcactgatagcctcttcaccatctcctctgtcctgcttaagtgctccatgtgtctggaatgtttaacttggagtaactactcactgacttggagaccacctgttctactttgagaaatcagaactgttctgtggatgcactgacagcgtgctccaactgcatatgcacccaggtttgtcaggagcatggaaggaaacctgcatctccctgtttactgggcccaaacctgaaagggtcttaagctgcagacagcttctcagtagcacagagctgaaggctttttgaaccaggagtctgggttgtggcttgggtcgcagtaagggcttagcctatcaatgcagaattcacattgaaaaagactttcctctcttgtcccaacacaaaaaagcaagccaagatctgatgcccatatcactgcctcctctgacttgggctacaggagtttcctgaaggaaaccaaattttacatctctgtcacattccagatcaccttagaggccacgctcccaagattagttatcaccctggcagtatgaatacttccctaaggcctcccatccatggaggggaagagtgggaaccagctgttacactcagcatctactgagcactgatgggagccctgcctgggccatgtgctgtggggccaaatggacatcactccctaacttcttgaggtctgtctcctctgtggattcacgcatgtatcaacctcattaaactatgccaaacttttgcctcc

SEQ ID NO: 2 - protein, 404 aa, Homo sapiens
  #human GPR182 protein (NCBI Accession ID.: AAH34761.1)
MSVKPSWGPGPSEGVTAVPTSDLGEIHNWTELLDLFNHTLSECHVELSQSTKRVVLFALYLAMFVVGLVENLLVICVNWRGSGRAGLMNLYILNMAIADLGIVLSLPVWMLEVTLDYTWLWGSFSCRFTHYFYFVNMYSSIFFLVCLSVDRYVTLTSASPSWQRYQHRVRRAMCAGIWVLSAIIPLPEVVHIQLVEGPEPMCLFMAPFETYSTWALAVALSTTILGFLLPFPLITVFNVLTACRLRQPGQPKSRRHCLLLCAYVAVFVMCWLPYHVTLLLLTLHGTHISLHCHLVHLLYFFYDVIDCFSMLHCVINPILYNFLSPHFRGRLLNAVVHYLPKDQTKAGTCASSSSCSTQHSIIITKGDSQPAAAAPHPEPSLSFQAHHLLPNTSPISPTQPLTPS

SEQ ID NO: 3 - protein, 404 aa, Homo sapiens [sequence omitted]